European Patent Specification EP 4 348 257 B1, published February 4, 2026. Title: METHODS FOR MODULATING HOST CELL SURFACE INTERACTIONS WITH HUMAN CYTOMEGALOVIRUS. Applicant: Genentech, Inc. The sequence listing filed with the application follows.

SEQUENCE LISTING (8 sequences)

SEQ ID NO: 1 - protein, 742 aa, Human cytomegalovirus
MRPGLPSYLIILAVCLFSHLLSSRYGAEAVSEPLDKAFHLLLNTYGRPIRFLRENTTQCTYNSSLRNSTVVRENAISFNFFQSYNQYYVFHMPRCLFAGPLAEQFLNQVDLTETLERYQQRLNTYALVSKDLASYRSFSQQLKAQDSLGEQPTTVPPPIDLSIPHVWMPPQTTPHGWTESHTTSGLHRPHFNQTCILFDGHDLLFSTVTPCLHQGFYLIDELRYVKITLTEDFFVVTVSIDDDTPMLLIFGHLPRVLFKAPYQRDNFILRQTEKHELLVLVKKDQLNRHSYLKDPDFLDAALDFNYLDLSALLRNSFHRYAVDVLKSGRCQMLDRRTVEMAFAYALALFAAARQEEAGAQVSVPRALDRQAALLQIQEFMITCLSQTPPRTTLLLYPTAVDLAKRALWTPNQITDITSLVRLVYILSKQNQQHLIPQWALRQIADFALKLHKTHLASFLSAFARQELYLMGSLVHSMLVHTTERREIFIVETGLCSLAELSHFTQLLAHPHHEYLSDLYTPCSSSGRRDHSLERLTRLFPDATVPATVPAALSILSTMQPSTLETFPDLFCLPLGESFSALTVSEHVSYIVTNQYLIKGISYPVSTTVVGQSLIITQTDSQTKCELTRNMHTTHSITVALNISLENCAFCQSALLEYDDTQGVINIMYMHDSDDVLFALDPYNEVVVSSPRTHYLMLLKNGTVLEVTDVVVDATDSRLLMMSVYALSAIIGIYLLYRMLKTC

SEQ ID NO: 2 - protein, 278 aa, Human cytomegalovirus
MCRRPDCGFSFSPGPVILLWCCLLLPIVSSAAVSVAPTAAEKVPAECPELTRRCLLGEVFEGDKYESWLRPLVNVTGRDGPLSQLIRYRPVTPEAANSVLLDEAFLDTLALLYNNPDQLRALLTLLSSDTAPRWMTVMRGYSECGDGSPAVYTCVDDLCRGYDLTRLSYGRSIFTEHVLGFELVPPSLFNVVVAIRNEATRTNRAVRLPVSTAAAPEGITLFYGLYNAVKEFCLRHQLDPPLLRHLDKYYAGLPPELKQTRVNLPAHSRYGPQAVDAR

SEQ ID NO: 3 - protein, 171 aa, Human cytomegalovirus
MSPKNLTPFLTALWLLLDHSRVPRVRAEECCEFINVNHPPERCYDFKMCNRFTVALRCPDGEVCYSPEKTAEIRGIVTTMTHSLTRQVVHNKLTSCNYNPLYLEADGRIRCGKVNDKAQYLLGAAGSVPYRWINLEYDKITRIVGLNQYLESVKKHKRLDVCRAKMGYMLQ

SEQ ID NO: 4 - protein, 214 aa, Human cytomegalovirus
MLRLLLRHHFHCLLLCAVWATPCLASPWSTLTANQNPSPPWSKLTYSKPHDAATFYCPFLYPSPPRSPLQFSGFQRVSTGPECRNETLYLLYNREGQTLVERSSTWVKKVIWYLSGRNQTILQRMPRTASKPSDGNVQISVEDAKIFGAHMVPKQTKLLRFVVNDGTRYQMCVMKLESWAHVFRDYSVSFQVRLTFTEANNQTYTFCTHPNLIV

SEQ ID NO: 5 - protein, 129 aa, Human cytomegalovirus
MRLCRVWLSVCLCAVVLGQCQRETAEKNDYYRVPHYWDACSRALPDQTRYKYVEQLVDLTLNYHYDASHGLDNFDVLKRINVTEVSLLISDFRRQNRRGGTNKRTTFNAAGSLAPHARSLEFSVRLFAN

SEQ ID NO: 6 - protein, 590 aa, Homo sapiens
MERGLPLLCAVLALVLAPAGAFRNDKCGDTIKIESPGYLTSPGYPHSYHPSEKCEWLIQAPDPYQRIMINFNPHFDLEDRDCKYDYVEVFDGENENGHFRGKFCGKIAPPPVVSSGPFLFIKFVSDYETHGAGFSIRYEIFKRGPECSQNYTTPSGVIKSPGFPEKYPNSLECTYIVFVPKMSEIILEFESFDLEPDSNPPGGMFCRYDRLEIWDGFPDVGPHIGRYCGQKTPGRIRSSSGILSMVFYTDSAIAKEGFSANYSVLQSSVSEDFKCMEALGMESGEIHSDQITASSQYSTNWSAERSRLNYPENGWTPGEDSYREWIQVDLGLLRFVTAVGTQGAISKETKKKYYVKTYKIDVSSNGEDWITIKEGNKPVLFQGNTNPTDVVVAVFPKPLITRFVRIKPATWETGISMRFEVYGCKITDYPCSGMLGMVSGLISDSQITSSNQGDRNWMPENIRLVTSRSGWALPPAPHSYINEWLQIDLGEEKIVRGIIIQGGKHRENKVFMRKFKIGYSNNGSDWKMIMDDSKRKAKSFEGNNNYDTPELRTFPALSTRFIRIYPERATHGGLGLRMELLGCEVEAPTA

SEQ ID NO: 7 - protein, 599 aa, Homo sapiens
MDMFPLTWVFLALYFSRHQVRGQPDPPCGGRLNSKDAGYITSPGYPQDYPSHQNCEWIVYAPEPNQKIVLNFNPHFEIEKHDCKYDFIEIRDGDSESADLLGKHCGNIAPPTIISSGSMLYIKFTSDYARQGAGFSLRYEIFKTGSEDCSKNFTSPNGTIESPGFPEKYPHNLDCTFTILAKPKMEIILQFLIFDLEHDPLQVGEGDCKYDWLDIWDGIPHVGPLIGKYCGTKTPSELRSSTGILSLTFHTDMAVAKDGFSARYYLVHQEPLENFQCNVPLGMESGRIANEQISASSTYSDGRWTPQQSRLHGDDNGWTPNLDSNKEYLQVDLRFLTMLTAIATQGAISRETQNGYYVKSYKLEVSTNGEDWMVYRHGKNHKVFQANNDATEVVLNKLHAPLLTRFVRIRPQTWHSGIALRLELFGCRVTDAPCSNMLGMLSGLIADSQISASSTQEYLWSPSAARLVSSRSGWFPRIPQAQPGEEWLQVDLGTPKTVKGVIIQGARGGDSITAVEARAFVRKFKVSYSLNGKDWEYIQDPRTQQPKLFEGNMHYDTPDIRRFDPIPAQYVRVYPERWSPAGIGMRLEVLGCDWTDSKP

SEQ ID NO: 8 - RNA, 20 nt, Artificial Sequence
  Synthetic Construct
gggtagtcctgggggtaacc